European Patent Specification EP 3 509 619 B1, published June 26, 2024. Title: PEPTIDES AND PEPTIDE CONJUGATES FOR TREATING MENTAL DISORDERS. Applicant: Kyoto University KAZUSA DNA RESEARCH INSTITUTE. The sequence listing filed with the application follows.

SEQUENCE LISTING (44 sequences)

SEQ ID NO: 1 - protein, 10 aa, Artificial Sequence
  Designed peptide
LSSTQAQQSY

SEQ ID NO: 2 - protein, 9 aa, Artificial Sequence
  Designed peptide
LSSTQAQQS

SEQ ID NO: 3 - protein, 9 aa, Artificial Sequence
  Designed peptide
SSTQAQQSY

SEQ ID NO: 4 - protein, 5 aa, Artificial Sequence
  Designed peptide
LSSTQ

SEQ ID NO: 5 - protein, 5 aa, Artificial Sequence
  Designed peptide
AQQSY

SEQ ID NO: 6 - protein, 10 aa, Artificial Sequence
  Designed peptide
LSSTQAQQSW

SEQ ID NO: 7 - protein, 10 aa, Artificial Sequence
  Designed peptide
LSSTQAQQSF

SEQ ID NO: 8 - protein, 5 aa, Artificial Sequence
  Designed peptide
SSTQA

SEQ ID NO: 9 - protein, 5 aa, Artificial Sequence
  Designed peptide
STQAQ

SEQ ID NO: 10 - protein, 5 aa, Artificial Sequence
  Designed peptide
TQAQQ

SEQ ID NO: 11 - protein, 5 aa, Artificial Sequence
  Designed peptide
QAQQS

SEQ ID NO: 12 - protein, 5 aa, Artificial Sequence
  Designed peptide
AQQSW

SEQ ID NO: 13 - protein, 5 aa, Artificial Sequence
  Designed peptide
AQQSF

SEQ ID NO: 14 - protein, 6 aa, Artificial Sequence
  Designed peptide
LSSTQA

SEQ ID NO: 15 - protein, 6 aa, Artificial Sequence
  Designed peptide
SSTQAQ

SEQ ID NO: 16 - protein, 6 aa, Artificial Sequence
  Designed peptide
STQAQQ

SEQ ID NO: 17 - protein, 6 aa, Artificial Sequence
  Designed peptide
TQAQQS

SEQ ID NO: 18 - protein, 6 aa, Artificial Sequence
  Designed peptide
QAQQSY

SEQ ID NO: 19 - protein, 6 aa, Artificial Sequence
  Designed peptide
QAQQSW

SEQ ID NO: 20 - protein, 6 aa, Artificial Sequence
  Designed peptide
QAQQSF

SEQ ID NO: 21 - protein, 7 aa, Artificial Sequence
  Designed peptide
LSSTQAQ

SEQ ID NO: 22 - protein, 7 aa, Artificial Sequence
  Designed peptide
SSTQAQQ

SEQ ID NO: 23 - protein, 7 aa, Artificial Sequence
  Designed peptide
STQAQQS

SEQ ID NO: 24 - protein, 7 aa, Artificial Sequence
  Designed peptide
TQAQQSY

SEQ ID NO: 25 - protein, 7 aa, Artificial Sequence
  Designed peptide
TQAQQSW

SEQ ID NO: 26 - protein, 7 aa, Artificial Sequence
  Designed peptide
TQAQQSF

SEQ ID NO: 27 - protein, 8 aa, Artificial Sequence
  Designed peptide
LSSTQAQQ

SEQ ID NO: 28 - protein, 8 aa, Artificial Sequence
  Designed peptide
SSTQAQQS

SEQ ID NO: 29 - protein, 8 aa, Artificial Sequence
  Designed peptide
STQAQQSY

SEQ ID NO: 30 - protein, 8 aa, Artificial Sequence
  Designed peptide
STQAQQSW

SEQ ID NO: 31 - protein, 8 aa, Artificial Sequence
  Designed peptide
STQAQQSF

SEQ ID NO: 32 - protein, 9 aa, Artificial Sequence
  Designed peptide
SSTQAQQSW

SEQ ID NO: 33 - protein, 9 aa, Artificial Sequence
  Designed peptide
SSTQAQQSF

SEQ ID NO: 34 - protein, 10 aa, Artificial Sequence
  Designed peptide
  MISC_FEATURE (10)..(10): Xaa(10)=Y, W, or F
LSSTQAQQSX

SEQ ID NO: 35 - protein, 30 aa, Artificial Sequence
  Designed peptide
  MISC_FEATURE (20)..(20): Xaa(20)=Y, W, or F
NKPGRFESFFLSSTQAQQSXLQGFSKNILE

SEQ ID NO: 36 - protein, 10 aa, Artificial Sequence
  Designed peptide
  MOD_RES (10)..(10): Carboxyl group of the C-terminus is amidated.
LSSTQAQQSY

SEQ ID NO: 37 - protein, 11 aa, Artificial Sequence
  Designed peptide
LSSTQAQQSYW

SEQ ID NO: 38 - protein, 11 aa, Artificial Sequence
  Designed peptide
WLSSTQAQQSY

SEQ ID NO: 39 - protein, 12 aa, Artificial Sequence
  Designed peptide
WLSSTQAQQSYW

SEQ ID NO: 40 - protein, 6 aa, Artificial Sequence
  Designed peptide
WLSSTQ

SEQ ID NO: 41 - protein, 6 aa, Artificial Sequence
  Designed peptide
AQQSYW

SEQ ID NO: 42 - protein, 14 aa, Artificial Sequence
  Designed peptide
ESFFLSSTQAQQSY

SEQ ID NO: 43 - protein, 14 aa, Artificial Sequence
  Designed peptide
LSSTQAQQSYLQGF

SEQ ID NO: 44 - protein, 14 aa, Artificial Sequence
  Designed peptide
FFLSSTQAQQSYLQ